European Patent Application EP 4 434 998 A1, published September 25, 2024. Title: 一种IL-15突变体融合蛋白药物组合物. Applicant: 江苏先声药业有限公司. Application CN. The sequence listing filed with the application follows.

SEQUENCE LISTING (26 sequences)

SEQ ID NO: 1 - protein, 114 aa, Homo sapiens
NWVNVISDLKKIEDLIQSMHIDATLYTESDVHPSCKVTAMKCFLLELQVISLESGDASIHDTVENLIILANNSLSSNGNVTESGCKECEELEEKNIKEFLQSFVHIVQMFINTS

SEQ ID NO: 2 - protein, 114 aa, synthetic construct
NWVNVISSLKKIEDLIQSMHIDATLYTESDVHPSCKVTAMKCFLLELQVISLESGDASIHDTVENLIILANNSLSSNGNVTESGCKECEELEEKNIKEFLQSFVHIVQMFINTS

SEQ ID NO: 3 - protein, 114 aa, synthetic construct
NWVNVISDLKKIEDLIQSMHIDATLYTESDVHPSCKVTAMKCFLLELQVISLESGDASIHDTVENLIILANNSLSSNGNVTESGCKECEELEEKNIKEFLQSFVKIVQMFINTS

SEQ ID NO: 4 - protein, 114 aa, synthetic construct
NWVNVISGLKKIEDLIQSMHIDATLYTESDVHPSCKVTAMKCFLLELQVISLESGDASIHDTVENLIILANNSLSSNGNVTESGCKECEELEEKNIKEFLQSFVHIVQMFINTS

SEQ ID NO: 5 - protein, 114 aa, synthetic construct
NWVNVISSLKKIEDLIQSMHIDATLYTESDVHPSCKVTAMKCFLLELQVISLESGDASIHDTVENLIILANNSLSSNGNVTESGCKECEELEEKNIKEFLQSFVKIVQMFINTS

SEQ ID NO: 6 - protein, 114 aa, synthetic construct
NWLNVISELKKIEDLIQSMHIDATLYTESDVHPSCKVTAMKCFLLELQVISLESGDASIHDTVENLIILANNSLSSNGNVTESGCKECEELEEKNIKEFLQSFVHIVQMFINTS

SEQ ID NO: 7 - protein, 114 aa, synthetic construct
NWLNVDSDLKKIEDLIQSMHIDATLYTESDVHPSCKVTAMKCFLLELQVISLESGDASIHDTVENLIILANNSLSSNGNVTESGCKECEELEEKNIKEFLQSFVHIVQMFINTS

SEQ ID NO: 8 - protein, 75 aa, synthetic construct
CPPPMSVEHADIWVKSYSLYSRERYICNSGFKRKAGTSSLTECVLNKATNVAHWTTPSLKCIRDPALVHQRPAPP

SEQ ID NO: 9 - protein, 63 aa, synthetic construct
CPPPMSVEHADIWVKSYSLYSRERYICNSGFKRKAGTSSLTECVLNKATNVAHWTTPSLKCIR

SEQ ID NO: 10 - protein, 77 aa, synthetic construct
ITCPPPMSVEHADIWVKSYSLYSRERYICNSGFKRKAGTSSLTECVLNKATNVAHWTTPSLKCIRDPALVHQRPAPP

SEQ ID NO: 11 - protein, 65 aa, synthetic construct
ITCPPPMSVEHADIWVKSYSLYSRERYICNSGFKRKAGTSSLTECVLNKATNVAHWTTPSLKCIR

SEQ ID NO: 12 - protein, 232 aa, synthetic construct
EPKSSDKTHTCPPCPAPEAAGGPSVFLFPPKPKDTLMISRTPEVTCVVVDVSHEDPEVKFNWYVDGVEVHNAKTKPREEQYNSTYRVVSVLTVLHQDWLNGKEYKCKVSNKALPAPIEKTISKAKGQPREPQVYTLPPSREEMTKNQVSLTCLVKGFYPSDIAVEWESNGQPENNYKTTPPVLDSDGSFFLYSKLTVDKSRWQQGNVFSCSVMHEALHNHYTQKSLSLSPGK

SEQ ID NO: 13 - protein, 20 aa, synthetic construct
SGGSGGGGSGGGSGGGGSLQ

SEQ ID NO: 14 - protein, 15 aa, synthetic construct
GGGGSGGGGSGGGGS

SEQ ID NO: 15 - skipped

SEQ ID NO: 16 - protein, 26 aa, synthetic construct
SGGGSGGGGSGGGGSGGGGSGGGSLQ

SEQ ID NO: 17 - protein, 448 aa, synthetic construct
EVQLVESGGGLVQPGGSLRLSCAASGFTFSDSWIHWVRQAPGKGLEWVAWISPYGGSTYYADSVKGRFTISADTSKNTAYLQMNSLRAEDTAVYYCARRHWPGGFDYWGQGTLVTVSSASTKGPSVFPLAPSSKSTSGGTAALGCLVKDYFPEPVTVSWNSGALTSGVHTFPAVLQSSGLYSLSSVVTVPSSSLGTQTYICNVNHKPSNTKVDKKVEPKSCDKTHTCPPCPAPELLGGPSVFLFPPKPKDTLMISRTPEVTCVVVDVSHEDPEVKFNWYVDGVEVHNAKTKPREEQYNSTYRVVSVLTVLHQDWLNGKEYKCKVSNKALPAPIEKTISKAKGQPREPQVYTLPPSREEMTKNQVSLTCLVKGFYPSDIAVEWESNGQPENNYKTTPPVLDSDGSFFLYSKLTVDKSRWQQGNVFSCSVMHEALHNHYTQKSLSLSPGK

SEQ ID NO: 18 - protein, 214 aa, synthetic construct
DIQMTQSPSSLSASVGDRVTITCRASQDVSTAVAWYQQKPGKAPKLLIYSASFLYSGVPSRFSGSGSGTDFTLTISSLQPEDFATYYCQQYLYHPATFGQGTKVEIKRTVAAPSVFIFPPSDEQLKSGTASVVCLLNNFYPREAKVQWKVDNALQSGNSQESVTEQDSKDSTYSLSSTLTLSKADYEKHKVYACEVTHQGLSSPVTKSFNRGEC

SEQ ID NO: 19 - protein, 448 aa, synthetic construct
QVQLQQSGPGLVKPSQTLSLTCAVSGDSITSGYWNWIRKFPSRGLEYMGYISYSGSTYYNPFLKSRISINRDTSKNQYYLQLNSVTPEDTAVYYCAKMGDWLAWFAYWGQGTLVTVSSASTKGPSVFPLAPSSKSTSGGTAALGCLVKDYFPEPVTVSWNSGALTSGVHTFPAVLQSSGLYSLSSVVTVPSSSLGTQTYICNVNHKPSNTKVDKKVEPKSCDKTHTCPPCPAPELLGGPSVFLFPPKPKDTLMISRTPEVTCVVVDVSHEDPEVKFNWYVDGVEVHNAKTKPREEQYNSTYRVVSVLTVLHQDWLNGKEYKCKVSNKALPAPIEKTISKAKGQPREPQVYTLPPSREEMTKNQVSLTCLVKGFYPSDIAVEWESNGQPENNYKTTPPVLDSDGSFFLYSKLTVDKSRWQQGNVFSCSVMHEALHNHYTQKSLSLSPGK

SEQ ID NO: 20 - protein, 448 aa, synthetic construct
QVQLQQSGPGLVKPSQTLSLTCAVSGDSITSGYWNWIRKFPSRGLEYMGYISYSGSTYYNPFLKSRISINRDTSKNQYYLQLNSVTPEDTAVYYCAKMGDWLAWFAYWGQGTLVTVSSASTKGPSVFPLAPSSKSTSGGTAALGCLVKDYFPEPVTVSWNSGALTSGVHTFPAVLQSSGLYSLSSVVTVPSSSLGTQTYICNVNHKPSNTKVDKKVEPKSCDKTHTCPPCPAPEAAGGPSVFLFPPKPKDTLMISRTPEVTCVVVDVSHEDPEVKFNWYVDGVEVHNAKTKPREEQYNSTYRVVSVLTVLHQDWLNGKEYKCKVSNKALPAPIEKTISKAKGQPREPQVYTLPPSREEMTKNQVSLTCLVKGFYPSDIAVEWESNGQPENNYKTTPPVLDSDGSFFLYSKLTVDKSRWQQGNVFSCSVMHEALHNHYTQKSLSLSPGK

SEQ ID NO: 21 - protein, 220 aa, synthetic construct
EIVMTQSPPTLSLSPGERVTLSCKSSQSLLYSSNQKNSLAWYQQKPGQAPRLLIYWASTRESGIPARFSGSGSGTDFTLTISSLQPEDFAVYYCQQYYGYPYTFGQGTKLEIKRTVAAPSVFIFPPSDEQLKSGTASVVCLLNNFYPREAKVQWKVDNALQSGNSQESVTEQDSKDSTYSLSSTLTLSKADYEKHKVYACEVTHQGLSSPVTKSFNRGEC

SEQ ID NO: 22 - protein, 657 aa, synthetic construct
QVQLQQSGPGLVKPSQTLSLTCAVSGDSITSGYWNWIRKFPSRGLEYMGYISYSGSTYYNPFLKSRISINRDTSKNQYYLQLNSVTPEDTAVYYCAKMGDWLAWFAYWGQGTLVTVSSASTKGPSVFPLAPSSKSTSGGTAALGCLVKDYFPEPVTVSWNSGALTSGVHTFPAVLQSSGLYSLSSVVTVPSSSLGTQTYICNVNHKPSNTKVDKKVEPKSCDKTHTCPPCPAPELLGGPSVFLFPPKPKDTLMISRTPEVTCVVVDVSHEDPEVKFNWYVDGVEVHNAKTKPREEQYNSTYRVVSVLTVLHQDWLNGKEYKCKVSNKALPAPIEKTISKAKGQPREPQVYTLPPSREEMTKNQVSLTCLVKGFYPSDIAVEWESNGQPENNYKTTPPVLDSDGSFFLYSKLTVDKSRWQQGNVFSCSVMHEALHNHYTQKSLSLSPGSCPPPMSVEHADIWVKSYSLYSRERYICNSGFKRKAGTSSLTECVLNKATNVAHWTTPSLKCIRDPALVHQRPAPPSGGSGGGGSGGGSGGGGSLQNWVNVISSLKKIEDLIQSMHIDATLYTESDVHPSCKVTAMKCFLLELQVISLESGDASIHDTVENLIILANNSLSSNGNVTESGCKECEELEEKNIKEFLQSFVKIVQMFINTS

SEQ ID NO: 23 - protein, 657 aa, synthetic construct
QVQLQQSGPGLVKPSQTLSLTCAVSGDSITSGYWNWIRKFPSRGLEYMGYISYSGSTYYNPFLKSRISINRDTSKNQYYLQLNSVTPEDTAVYYCAKMGDWLAWFAYWGQGTLVTVSSASTKGPSVFPLAPSSKSTSGGTAALGCLVKDYFPEPVTVSWNSGALTSGVHTFPAVLQSSGLYSLSSVVTVPSSSLGTQTYICNVNHKPSNTKVDKKVEPKSCDKTHTCPPCPAPEAAGGPSVFLFPPKPKDTLMISRTPEVTCVVVDVSHEDPEVKFNWYVDGVEVHNAKTKPREEQYNSTYRVVSVLTVLHQDWLNGKEYKCKVSNKALPAPIEKTISKAKGQPREPQVYTLPPSREEMTKNQVSLTCLVKGFYPSDIAVEWESNGQPENNYKTTPPVLDSDGSFFLYSKLTVDKSRWQQGNVFSCSVMHEALHNHYTQKSLSLSPGSCPPPMSVEHADIWVKSYSLYSRERYICNSGFKRKAGTSSLTECVLNKATNVAHWTTPSLKCIRDPALVHQRPAPPSGGSGGGGSGGGSGGGGSLQNWVNVISSLKKIEDLIQSMHIDATLYTESDVHPSCKVTAMKCFLLELQVISLESGDASIHDTVENLIILANNSLSSNGNVTESGCKECEELEEKNIKEFLQSFVKIVQMFINTS

SEQ ID NO: 24 - protein, 657 aa, synthetic construct
QVQLQQSGPGLVKPSQTLSLTCAVSGDSITSGYWNWIRKFPSRGLEYMGYISYSGSTYYNPFLKSRISINRDTSKNQYYLQLNSVTPEDTAVYYCAKMGDWLAWFAYWGQGTLVTVSSASTKGPSVFPLAPSSKSTSGGTAALGCLVKDYFPEPVTVSWNSGALTSGVHTFPAVLQSSGLYSLSSVVTVPSSSLGTQTYICNVNHKPSNTKVDKKVEPKSCDKTHTCPPCPAPELLGGPSVFLFPPKPKDTLMISRTPEVTCVVVDVSHEDPEVKFNWYVDGVEVHNAKTKPREEQYNSTYRVVSVLTVLHQDWLNGKEYKCKVSNKALPAPIEKTISKAKGQPREPQVYTLPPSREEMTKNQVSLTCLVKGFYPSDIAVEWESNGQPENNYKTTPPVLDSDGSFFLYSKLTVDKSRWQQGNVFSCSVMHEALHNHYTQKSLSLSPGSCPPPMSVEHADIWVKSYSLYSRERYICNSGFKRKAGTSSLTECVLNKATNVAHWTTPSLKCIRDPALVHQRPAPPSGGSGGGGSGGGSGGGGSLQNWLNVISELKKIEDLIQSMHIDATLYTESDVHPSCKVTAMKCFLLELQVISLESGDASIHDTVENLIILANNSLSSNGNVTESGCKECEELEEKNIKEFLQSFVHIVQMFINTS

SEQ ID NO: 25 - protein, 657 aa, synthetic construct
QVQLQQSGPGLVKPSQTLSLTCAVSGDSITSGYWNWIRKFPSRGLEYMGYISYSGSTYYNPFLKSRISINRDTSKNQYYLQLNSVTPEDTAVYYCAKMGDWLAWFAYWGQGTLVTVSSASTKGPSVFPLAPSSKSTSGGTAALGCLVKDYFPEPVTVSWNSGALTSGVHTFPAVLQSSGLYSLSSVVTVPSSSLGTQTYICNVNHKPSNTKVDKKVEPKSCDKTHTCPPCPAPELLGGPSVFLFPPKPKDTLMISRTPEVTCVVVDVSHEDPEVKFNWYVDGVEVHNAKTKPREEQYNSTYRVVSVLTVLHQDWLNGKEYKCKVSNKALPAPIEKTISKAKGQPREPQVYTLPPSREEMTKNQVSLTCLVKGFYPSDIAVEWESNGQPENNYKTTPPVLDSDGSFFLYSKLTVDKSRWQQGNVFSCSVMHEALHNHYTQKSLSLSPGSCPPPMSVEHADIWVKSYSLYSRERYICNSGFKRKAGTSSLTECVLNKATNVAHWTTPSLKCIRDPALVHQRPAPPSGGSGGGGSGGGSGGGGSLQNWLNVDSDLKKIEDLIQSMHIDATLYTESDVHPSCKVTAMKCFLLELQVISLESGDASIHDTVENLIILANNSLSSNGNVTESGCKECEELEEKNIKEFLQSFVHIVQMFINTS

SEQ ID NO: 26 - protein, 657 aa, synthetic construct
QVQLQQSGPGLVKPSQTLSLTCAVSGDSITSGYWNWIRKFPSRGLEYMGYISYSGSTYYNPFLKSRISINRDTSKNQYYLQLNSVTPEDTAVYYCAKMGDWLAWFAYWGQGTLVTVSSASTKGPSVFPLAPSSKSTSGGTAALGCLVKDYFPEPVTVSWNSGALTSGVHTFPAVLQSSGLYSLSSVVTVPSSSLGTQTYICNVNHKPSNTKVDKKVEPKSCDKTHTCPPCPAPELLGGPSVFLFPPKPKDTLMISRTPEVTCVVVDVSHEDPEVKFNWYVDGVEVHNAKTKPREEQYNSTYRVVSVLTVLHQDWLNGKEYKCKVSNKALPAPIEKTISKAKGQPREPQVYTLPPSREEMTKNQVSLTCLVKGFYPSDIAVEWESNGQPENNYKTTPPVLDSDGSFFLYSKLTVDKSRWQQGNVFSCSVMHEALHNHYTQKSLSLSPGSCPPPMSVEHADIWVKSYSLYSRERYICNSGFKRKAGTSSLTECVLNKATNVAHWTTPSLKCIRDPALVHQRPAPPSGGSGGGGSGGGSGGGGSLQNWVNVISDLKKIEDLIQSMHIDATLYTESDVHPSCKVTAMKCFLLELQVISLESGDASIHDTVENLIILANNSLSSNGNVTESGCKECEELEEKNIKEFLQSFVHIVQMFINTS